European Patent Application EP 4 520 825 A1, published March 12, 2025. Title: Artificial RNA molecule. Applicant: 学校法人常翔学園. Application WO. The sequence listing filed with the application follows.

SEQUENCE LISTING (42 sequences)

SEQ ID NO: 1 - skipped

SEQ ID NO: 2 - RNA, 32 nt, Mus musculus
  source 1..32: mol_type = transcribed RNA
gccggtagtggtggcgcacgccggtaggattt

SEQ ID NO: 3 - DNA, 21 bp, synthetic construct
  misc_feature 1..21: note = PCR primer
  source 1..21: mol_type = other DNA
tgaccgccaggattgagatac

SEQ ID NO: 4 - DNA, 20 bp, synthetic construct
  misc_feature 1..20: note = PCR primer
  source 1..20: mol_type = other DNA
tgatctggatcgccttttgc

SEQ ID NO: 5 - DNA, 22 bp, synthetic construct
  misc_feature 1..22: note = PCR primer
  source 1..22: mol_type = other DNA
tgggctcctacgattcttagag

SEQ ID NO: 6 - DNA, 22 bp, synthetic construct
  misc_feature 1..22: note = PCR primer
  source 1..22: mol_type = other DNA
gaaccagacaatgctcctgaag

SEQ ID NO: 7 - DNA, 22 bp, synthetic construct
  misc_feature 1..22: note = PCR primer
  source 1..22: mol_type = other DNA
ttctgagcaggagaatggtctg

SEQ ID NO: 8 - DNA, 22 bp, synthetic construct
  misc_feature 1..22: note = PCR primer
  source 1..22: mol_type = other DNA
catgggcatggagaaaactgag

SEQ ID NO: 9 - DNA, 682 bp, synthetic construct
  misc_feature 1..682: note = Slc40ex8.5 minigene
  source 1..682: mol_type = other DNA
ggatccactagtaacggccgccagtgtgctggaattcatctcttccgcatcgctgtctgcgagggccagctgttggggtgagtactccctctcaaaagcgggcatgacttctgcgctaagattgtcagtttccaaaaacgaggaggatttgatattcccctggcatacctatgcaacagttttctcatattgaactgctgattcatccaaatatcttaagtatatttctgagttttctaatttagtttaatttttgtggattcagggcctccctttgtaaccctggctgacctggaacttgatatattgaacaaactggcctcaaattcacagagatctgcctacctctgcctcctgagtgttaaaggtatgtgccattatgctcaacgaaaagtgaccttttttaaaaagtgattatagctaggtgtgatggctcatgtctgtaatagcaacatttgagagactgatgcctttgagggtggccgcgtccatctggtcagaaaagacaatctttttgttgtcaagcttgctgcacgtctagggcgcagtagtccagggtttccttgatgatgtcatacttatcctgtcccttttttttccacagctcgcggttgaggacaaactcttcgcggtctttccagtactcttggatcggaaacccgtcggcctccgaacgtctaga

SEQ ID NO: 10 - DNA, 662 bp, synthetic construct
  misc_feature 1..662: note = Smg6ex8.5 WT minigene
  source 1..662: mol_type = other DNA
ggatccactagtaacggccgccagtgtgctggaattcatctcttccgcatcgctgtctgcgagggccagctgttggggtgagtactccctctcaaaagcgggcatgacttctgcgctaagattgtcagtttccaaaaacgaggaggatttgatattcacctggcccggagagaactgaccctcattagttgtcttcagacgtccacacatgtatcatggtgtacattcattcattcattttcttttttttattgtttttgagacagcatctcatactgtagccccctggcctttaattcatgacaacccttctgcctctgacttctgggtaccaaattacaggtatgagttattatgtctaattcttttgggtttaatttaaaatttccatttgtcttcctatttccttcctattctgtaactgtctttgtggatgacttggggtgatgcctttgagggtggccgcgtccatctggtcagaaaagacaatctttttgttgtcaagcttgctgcacgtctagggcgcagtagtccagggtttccttgatgatgtcatacttatcctgtcccttttttttccacagctcgcggttgaggacaaactcttcgcggtctttccagtactcttggatcggaaacccgtcggcctccgaacgtctaga

SEQ ID NO: 11 - DNA, 682 bp, synthetic construct
  misc_feature 1..682: note = Slc25a40ex8.5 MUT minigene
  source 1..682: mol_type = other DNA
ggatccactagtaacggccgccagtgtgctggaattcatctcttccgcatcgctgtctgcgagggccagctgttggggtgagtactccctctcaaaagcgggcatgacttctgcgctaagattgtcagtttccaaaaacgaggaggatttgatattcccctggcatacctatgcaacagttttctcatattgaactgctgattcatccaaatatcttaagtatatttctgagttttctaatttagtttaatttttgtggattcagggcctccctttgtaagggtccgtgacctggaacttgatatattgaacaaactggcctcaaattcacagagatctgggtaggtgtcggtggtgagtgttaaaggtatgtgccattatgctcaacgaaaagtgaccttttttaaaaagtgattatagctaggtgtgatggctcatgtctgtaatagcaacatttgagagactgatgcctttgagggtggccgcgtccatctggtcagaaaagacaatctttttgttgtcaagcttgctgcacgtctagggcgcagtagtccagggtttccttgatgatgtcatacttatcctgtcccttttttttccacagctcgcggttgaggacaaactcttcgcggtctttccagtactcttggatcggaaacccgtcggcctccgaacgtctaga

SEQ ID NO: 12 - DNA, 56 bp, Homo sapiens
  source 1..56: mol_type = other DNA
ccaaacaattagtggaattggcaaaagaagaagacaaagccaccccaagttagatc

SEQ ID NO: 13 - DNA, 344 bp, synthetic construct
  misc_feature 1..344: note = FAS ex4-5-6 minigene
  source 1..344: mol_type = other DNA
gagggcctatttcccatgattccttcatatttgcatatacgatacaaggctgttagagagataattggaattaatttgactgtaaacacaaagatattagtacaaaatacgtgacgtagaaagtaataatttcttgggtagtttgcagttttaaaattatgttttaaaatggactatcatatgcttaccgtaacttgaaagtatttcgatttcttggctttatatatcttgtggaaaggacgaaacaccgccggtagtggtggcgcacgccggtaggatttccaaacaattagtggaattggcaaaagaagaagacaaagccaccccaagttagatcttttttt

SEQ ID NO: 14 - DNA, 1542 bp, synthetic construct
  misc_feature 1..1542: note = FAS ex5-6-7 minigene
  source 1..1542: mol_type = other DNA
ggatccgaacatggaatcatcaaggaatgcacactcaccagcaacaccaagtgcaaagaggaaggtaattatttttttacggttatattctcctttcccccaaccccatggaaagatgtgaagaaaaaccaatcactcttgattactagaaagtcctttatttaatcttaaagattgcttattttcatataaaatgtccaatgttccaacctacaggatccagatctaacttggggtggctttgtcttcttcttttgccaattccactaattgtttggggtaagttcttgctttgttcaaactgcagattgaaataacttgggaagtagttcacaaagatttgcctcattcttacctataaaaagctaccactttggtagatttatgtattgttaatttcttgcccctgaatgcagccttgagagctgactgataagaacaaatgaaattattcctcagctagtttctgagcaacagttttggggcattgagtggtattctcatccttcctatgaacaggtgttctctgcagcagcagaattggccaaaaatcagaagcaattcttcactattcattgagatctccctatgcaaaaagagaacacaagaagcaaaggcattcccaggaaacacattgcagggaacactttaaaaacttgtacttcactgcctcctcttcctcggcctaattgcttgtttttaattatttctccttcttaacttaaaatactatggggacacatgttatacaaaggtgacttagtagagtcagtagaaaagccaaaattagatattatcataattagtctagaaaaatccctttaagtcattcatcaactacagggtcacaccaactttcagtaacttagaagtattcaattttcccttctcagaacaattatctgtttcttcagttcagttgaagaagaaagtttgccttgcctttagcggttgtttagctgaaaatacatttgggatatttaagcactgtaattgtgctcagagacatacagattcttctatctcacattgactttaatgcatacacctattgagtatgtatgcttgagttatttgtgtgtgtatttcatttctgggcatccatagcaagttgatgttgacttgcttgtcctacggcttctgcatcctgccatagtcttgccgtccacatctttgctggacagagagtggtgcttgccatatggtaagtcaaaagccatctccttgctaggccagcctgtggtaattagatgactaattaagatatgtcctttcactagaacacttgacttagtagtacgaaagttccaaaatcagcggtctcctgcgatgtttggccacttttaagtttcactgaatttctcctttttccttcttatatttctcttagtgtgaaagtatgttctcacatgcattctacaaggctgagacctgagttgataaaatttctttgttctttcagtgaagagaaaggaagtacagaaaacatgcagaaagcacagaaaggaaaaccaaggttctcatgaatctccaactctcgag

SEQ ID NO: 15 - DNA, 30 bp, synthetic construct
  misc_feature 1..30: note = PCR primer
  source 1..30: mol_type = other DNA
gagctctctggctaactagagaacccactg

SEQ ID NO: 16 - DNA, 30 bp, synthetic construct
  misc_feature 1..30: note = PCR primer
  source 1..30: mol_type = other DNA
gctggcaactagaaggcacagtcgaggctg

SEQ ID NO: 17 - DNA, 56 bp, synthetic construct
  misc_feature 1..56: note = DMD ex53 #1
  source 1..56: mol_type = other DNA
cctccggttctgaaggtgttcttgtacttcatcccactgattctgaattctttcaa

SEQ ID NO: 18 - DNA, 56 bp, synthetic construct
  misc_feature 1..56: note = DMD ex53 #2
  source 1..56: mol_type = other DNA
cttagcttccagccattgtgttgaatcctttaacatttcattcaactgttgcctcc

SEQ ID NO: 19 - DNA, 56 bp, synthetic construct
  misc_feature 1..56: note = DMD ex53 #3
  source 1..56: mol_type = other DNA
ccatgactcaagcttggctctggcctgtcctaagacctgctcagcttcttccttag

SEQ ID NO: 20 - DNA, 56 bp, synthetic construct
  misc_feature 1..56: note = DMD ex53 #4
  source 1..56: mol_type = other DNA
cttggtttctgtgattttcttttggattgcatctactgtatagggaccctccttcc

SEQ ID NO: 21 - DNA, 344 bp, synthetic construct
  misc_feature 1..344: note = DMD ex53 #1
  source 1..344: mol_type = other DNA
gagggcctatttcccatgattccttcatatttgcatatacgatacaaggctgttagagagataattggaattaatttgactgtaaacacaaagatattagtacaaaatacgtgacgtagaaagtaataatttcttgggtagtttgcagttttaaaattatgttttaaaatggactatcatatgcttaccgtaacttgaaagtatttcgatttcttggctttatatatcttgtggaaaggacgaaacaccgccggtagtggtggcgcacgccggtaggatttcctccggttctgaaggtgttcttgtacttcatcccactgattctgaattctttcaattttttt

SEQ ID NO: 22 - DNA, 344 bp, synthetic construct
  misc_feature 1..344: note = DMD ex53 #2
  source 1..344: mol_type = other DNA
gagggcctatttcccatgattccttcatatttgcatatacgatacaaggctgttagagagataattggaattaatttgactgtaaacacaaagatattagtacaaaatacgtgacgtagaaagtaataatttcttgggtagtttgcagttttaaaattatgttttaaaatggactatcatatgcttaccgtaacttgaaagtatttcgatttcttggctttatatatcttgtggaaaggacgaaacaccgccggtagtggtggcgcacgccggtaggatttcttagcttccagccattgtgttgaatcctttaacatttcattcaactgttgcctccttttttt

SEQ ID NO: 23 - DNA, 344 bp, synthetic construct
  misc_feature 1..344: note = DMD ex53 #3
  source 1..344: mol_type = other DNA
gagggcctatttcccatgattccttcatatttgcatatacgatacaaggctgttagagagataattggaattaatttgactgtaaacacaaagatattagtacaaaatacgtgacgtagaaagtaataatttcttgggtagtttgcagttttaaaattatgttttaaaatggactatcatatgcttaccgtaacttgaaagtatttcgatttcttggctttatatatcttgtggaaaggacgaaacaccgccggtagtggtggcgcacgccggtaggatttccatgactcaagcttggctctggcctgtcctaagacctgctcagcttcttccttagttttttt

SEQ ID NO: 24 - DNA, 344 bp, synthetic construct
  misc_feature 1..344: note = DMD ex53 #4
  source 1..344: mol_type = other DNA
gagggcctatttcccatgattccttcatatttgcatatacgatacaaggctgttagagagataattggaattaatttgactgtaaacacaaagatattagtacaaaatacgtgacgtagaaagtaataatttcttgggtagtttgcagttttaaaattatgttttaaaatggactatcatatgcttaccgtaacttgaaagtatttcgatttcttggctttatatatcttgtggaaaggacgaaacaccgccggtagtggtggcgcacgccggtaggatttcttggtttctgtgattttcttttggattgcatctactgtatagggaccctccttccttttttt

SEQ ID NO: 25 - DNA, 798 bp, synthetic construct
  misc_feature 1..798: note = DMD ex53 minigene
  source 1..798: mol_type = other DNA
ggatccactagtaacggccgccagtgtgctggaattcatctcttccgcatcgctgtctgcgagggccagctgttggggtgagtactccctctcaaaagcgggcatgacttctgcgctaagattgtcagtttccaaaaacgaggaggatttgatattcacctggccctaagcaacataaatgtgagataacgtttggaagttacatttaaaatgtctcctccagactagcatttactactatatatttatttttccttttattctagttgaaagaattcagaatcagtgggatgaagtacaagaacaccttcagaaccggaggcaacagttgaatgaaatgttaaaggattcaacacaatggctggaagctaaggaagaagctgagcaggtcttaggacaggccagagccaagcttgagtcatggaaggagggtccctatacagtagatgcaatccaaaagaaaatcacagaaaccaaggttagtatcaaagatacctttttaaaataaaatactggttacatttgataaaattataccatagattgtaatttaatgatgtttaatgtaaagttattaaggtgatgcctttgagggtggccgcgtccatctggtcagaaaagacaatctttttgttgtcaagcttgctgcacgtctagggcgcagtagtccagggtttccttgatgatgtcatacttatcctgtcccttttttttccacagctcgcggttgaggacaaactcttcgcggtctttccagtactcttggatcggaaacccgtcggcctccgaacgtctaga

SEQ ID NO: 26 - DNA, 20 bp, synthetic construct
  misc_feature 1..20: note = PCR primer
  source 1..20: mol_type = other DNA
aagaccgcgaagagtttgtc

SEQ ID NO: 27 - DNA, 20 bp, synthetic construct
  misc_feature 1..20: note = PCR primer
  source 1..20: mol_type = other DNA
attcatctcttccgcatcgc

SEQ ID NO: 28 - DNA, 5801 bp, synthetic construct
  source 1..5801: mol_type = other DNA
gacggatcgggagatctcccgatcccctatggtgcactctcagtacaatctgctctgatgccgcatagttaagccagtatctgctccctgcttgtgtgttggaggtcgctgagtagtgcgcgagcaaaatttaagctacaacaaggcaaggcttgaccgacaattgcatgaagaatctgcttagggttaggcgttttgcgctgcttcgcgatgtacgggccagatatacgcgttgacattgattattgactagttattaatagtaatcaattacggggtcattagttcatagcccatatatggagttccgcgttacataacttacggtaaatggcccgcctggctgaccgcccaacgacccccgcccattgacgtcaataatgacgtatgttcccatagtaacgccaatagggactttccattgacgtcaatgggtggagtatttacggtaaactgcccacttggcagtacatcaagtgtatcatatgccaagtacgccccctattgacgtcaatgacggtaaatggcccgcctggcattatgcccagtacatgaccttatgggactttcctacttggcagtacatctacgtattagtcatcgctattaccatggtgatgcggttttggcagtacatcaatgggcgtggatagcggtttgactcacggggatttccaagtctccaccccattgacgtcaatgggagtttgttttggcaccaaaatcaacgggactttccaaaatgtcgtaacaactccgccccattgacgcaaatgggcggtaggcgtgtacggtgggaggtctatataagcagagctctctggctaactagagaacccactgcttactggcttatcgaaattaatacgactcactatagggagacccaagcttggtaccgagctcggatccactagtaacggccgccagtgtgctggaattcatctcttccgcatcgctgtctgcgagggccagctgttggggtgagtactccctctcaaaagcgggcatgacttctgcgctaagattgtcagtttccaaaaacgaggaggatttgatattcacctggcccgcggtgatgcctttgagggtggccgcgtccatctggtcagaaaagacaatctttttgttgtcaagcttgctgcacgtctagggcgcagtagtccagggtttccttgatgatgtcatacttatcctgtcccttttttttccacagctcgcggttgaggacaaactcttcgcggtctttccagtactcttggatcggaaacccgtcggcctccgaacgtctagactcgagcggccgccactgtgctggatatctgcagaattccaccacactggactagtggatccgagctcggtaccaagcttaagtttaaaccgctgatcagcctcgactgtgccttctagttgccagccatctgttgtttgcccctcccccgtgccttccttgaccctggaaggtgccactcccactgtcctttcctaataaaatgaggaaattgcatcgcattgtctgagtaggtgtcattctattctggggggtggggtggggcaggacagcaagggggaggattgggaagacaatagcaggcatgctggggatgcggtgggctctatggcttctgaggcggaaagaaccagctggggctctagggggtatccccacgcgccctgtagcggcgcattaagcgcggcgggtgtggtggttacgcgcagcgtgaccgctacacttgccagcgccctagcgcccgctcctttcgctttcttcccttcctttctcgccacgttcgccggctttccccgtcaagctctaaatcgggggctccctttagggttccgatttagtgctttacggcacctcgaccccaaaaaacttgattagggtgatggttcacgtagtgggccatcgccctgatagacggtttttcgccctttgacgttggagtccacgttctttaatagtggactcttgttccaaactggaacaacactcaaccctatctcggtctattcttttgatttataagggattttgccgatttcggcctattggttaaaaaatgagctgatttaacaaaaatttaacgcgaattaattctgtggaatgtgtgtcagttagggtgtggaaagtccccaggctccccagcaggcagaagtatgcaaagcatgcatctcaattagtcagcaaccaggtgtggaaagtccccaggctccccagcaggcagaagtatgcaaagcatgcatctcaattagtcagcaaccatagtcccgcccctaactccgcccatcccgcccctaactccgcccagttccgcccattctccgccccatggctgactaattttttttatttatgcagaggccgaggccgcctctgcctctgagctattccagaagtagtgaggaggcttttttggaggcctaggcttttgcaaaaagctcccgggagcttgtatatccattttcggatctgatcaagagacaggatgaggatcgtttcgcatgattgaacaagatggattgcacgcaggttctccggccgcttgggtggagaggctattcggctatgactgggcacaacagacaatcggctgctctgatgccgccgtgttccggctgtcagcgcaggggcgcccggttctttttgtcaagaccgacctgtccggtgccctgaatgaactgcaggacgaggcagcgcggctatcgtggctggccacgacgggcgttccttgcgcagctgtgctcgacgttgtcactgaagcgggaagggactggctgctattgggcgaagtgccggggcaggatctcctgtcatctcaccttgctcctgccgagaaagtatccatcatggctgatgcaatgcggcggctgcatacgcttgatccggctacctgcccattcgaccaccaagcgaaacatcgcatcgagcgagcacgtactcggatggaagccggtcttgtcgatcaggatgatctggacgaagagcatcaggggctcgcgccagccgaactgttcgccaggctcaaggcgcgcatgcccgacggcgaggatctcgtcgtgacccatggcgatgcctgcttgccgaatatcatggtggaaaatggccgcttttctggattcatcgactgtggccggctgggtgtggcggaccgctatcaggacatagcgttggctacccgtgatattgctgaagagcttggcggcgaatgggctgaccgcttcctcgtgctttacggtatcgccgctcccgattcgcagcgcatcgccttctatcgccttcttgacgagttcttctgagcgggactctggggttcgaaatgaccgaccaagcgacgcccaacctgccatcacgagatttcgattccaccgccgccttctatgaaaggttgggcttcggaatcgttttccgggacgccggctggatgatcctccagcgcggggatctcatgctggagttcttcgcccaccccaacttgtttattgcagcttataatggttacaaataaagcaatagcatcacaaatttcacaaataaagcatttttttcactgcattctagttgtggtttgtccaaactcatcaatgtatcttatcatgtctgtataccgtcgacctctagctagagcttggcgtaatcatggtcatagctgtttcctgtgtgaaattgttatccgctcacaattccacacaacatacgagccggaagcataaagtgtaaagcctggggtgcctaatgagtgagctaactcacattaattgcgttgcgctcactgcccgctttccagtcgggaaacctgtcgtgccagctgcattaatgaatcggccaacgcgcggggagaggcggtttgcgtattgggcgctcttccgcttcctcgctcactgactcgctgcgctcggtcgttcggctgcggcgagcggtatcagctcactcaaaggcggtaatacggttatccacagaatcaggggataacgcaggaaagaacatgtgagcaaaaggccagcaaaaggccaggaaccgtaaaaaggccgcgttgctggcgtttttccataggctccgcccccctgacgagcatcacaaaaatcgacgctcaagtcagaggtggcgaaacccgacaggactataaagataccaggcgtttccccctggaagctccctcgtgcgctctcctgttccgaccctgccgcttaccggatacctgtccgcctttctcccttcgggaagcgtggcgctttctcatagctcacgctgtaggtatctcagttcggtgtaggtcgttcgctccaagctgggctgtgtgcacgaaccccccgttcagcccgaccgctgcgccttatccggtaactatcgtcttgagtccaacccggtaagacacgacttatcgccactggcagcagccactggtaacaggattagcagagcgaggtatgtaggcggtgctacagagttcttgaagtggtggcctaactacggctacactagaagaacagtatttggtatctgcgctctgctgaagccagttaccttcggaaaaagagttggtagctcttgatccggcaaacaaaccaccgctggtagcggtttttttgtttgcaagcagcagattacgcgcagaaaaaaaggatctcaagaagatcctttgatcttttctacggggtctgacgctcagtggaacgaaaactcacgttaagggattttggtcatgagattatcaaaaaggatcttcacctagatccttttaaattaaaaatgaagttttaaatcaatctaaagtatatatgagtaaacttggtctgacagttaccaatgcttaatcagtgaggcacctatctcagcgatctgtctatttcgttcatccatagttgcctgactccccgtcgtgtagataactacgatacgggagggcttaccatctggccccagtgctgcaatgataccgcgagacccacgctcaccggctccagatttatcagcaataaaccagccagccggaagggccgagcgcagaagtggtcctgcaactttatccgcctccatccagtctattaattgttgccgggaagctagagtaagtagttcgccagttaatagtttgcgcaacgttgttgccattgctacaggcatcgtggtgtcacgctcgtcgtttggtatggcttcattcagctccggttcccaacgatcaaggcgagttacatgatcccccatgttgtgcaaaaaagcggttagctccttcggtcctccgatcgttgtcagaagtaagttggccgcagtgttatcactcatggttatggcagcactgcataattctcttactgtcatgccatccgtaagatgcttttctgtgactggtgagtactcaaccaagtcattctgagaatagtgtatgcggcgaccgagttgctcttgcccggcgtcaatacgggataataccgcgccacatagcagaactttaaaagtgctcatcattggaaaacgttcttcggggcgaaaactctcaaggatcttaccgctgttgagatccagttcgatgtaacccactcgtgcacccaactgatcttcagcatcttttactttcaccagcgtttctgggtgagcaaaaacaggaaggcaaaatgccgcaaaaaagggaataagggcgacacggaaatgttgaatactcatactcttcctttttcaatattattgaagcatttatcagggttattgtctcatgagcggatacatatttgaatgtatttagaaaaataaacaaataggggttccgcgcacatttccccgaaaagtgccacctgacgtc

SEQ ID NO: 29 - DNA, 25 bp, synthetic construct
  source 1..25: mol_type = other DNA
gccgggcatggtggcgcacgccttt

SEQ ID NO: 30 - DNA, 345 bp, synthetic construct
  source 1..345: mol_type = other DNA
gagggcctatttcccatgattccttcatatttgcatatacgatacaaggctgttagagagataattggaattaatttgactgtaaacacaaagatattagtacaaaatacgtgacgtagaaagtaataatttcttgggtagtttgcagttttaaaattatgttttaaaatggactatcatatgcttaccgtaacttgaaagtatttcgatttcttggctttatatatcttgtggaaaggacgaaacaccgccgggcatggtggcgcacgcctttaatcatttgctgaaggaggcagaggcaggaggatcacgagttcgaggccagcctgggctacacattttttt

SEQ ID NO: 31 - DNA, 56 bp, synthetic construct
  source 1..56: mol_type = other DNA
cttggtttctgtgatattctattggattgcatctactgtatagggaccctccttcc

SEQ ID NO: 32 - DNA, 344 bp, synthetic construct
  source 1..344: mol_type = other DNA
gagggcctatttcccatgattccttcatatttgcatatacgatacaaggctgttagagagataattggaattaatttgactgtaaacacaaagatattagtacaaaatacgtgacgtagaaagtaataatttcttgggtagtttgcagttttaaaattatgttttaaaatggactatcatatgcttaccgtaacttgaaagtatttcgatttcttggctttatatatcttgtggaaaggacgaaacaccgccggtagtggtggcgcacgccggtaggatttcttggtttctgtgatattctattggattgcatctactgtatagggaccctccttccttttttt

SEQ ID NO: 33 - DNA, 56 bp, synthetic construct
  source 1..56: mol_type = other DNA
aacatttcattcaactgttgcctccggttctgaaggtgttcttgtacttcatccca

SEQ ID NO: 34 - DNA, 344 bp, synthetic construct
  source 1..344: mol_type = other DNA
gagggcctatttcccatgattccttcatatttgcatatacgatacaaggctgttagagagataattggaattaatttgactgtaaacacaaagatattagtacaaaatacgtgacgtagaaagtaataatttcttgggtagtttgcagttttaaaattatgttttaaaatggactatcatatgcttaccgtaacttgaaagtatttcgatttcttggctttatatatcttgtggaaaggacgaaacaccgccggtagtggtggcgcacgccggtaggatttaacatttcattcaactgttgcctccggttctgaaggtgttcttgtacttcatcccattttttt

SEQ ID NO: 35 - DNA, 112 bp, synthetic construct
  source 1..112: mol_type = other DNA
cttggtttctgtgatattctattggattgcatctactgaatagggacccaccttccaacatttcattcaacagttgcctccggttcagaaggtgttcttgaacttcatccca

SEQ ID NO: 36 - DNA, 400 bp, synthetic construct
  source 1..400: mol_type = other DNA
gagggcctatttcccatgattccttcatatttgcatatacgatacaaggctgttagagagataattggaattaatttgactgtaaacacaaagatattagtacaaaatacgtgacgtagaaagtaataatttcttgggtagtttgcagttttaaaattatgttttaaaatggactatcatatgcttaccgtaacttgaaagtatttcgatttcttggctttatatatcttgtggaaaggacgaaacaccgccggtagtggtggcgcacgccggtaggatttcttggtttctgtgatattctattggattgcatctactgaatagggacccaccttccaacatttcattcaacagttgcctccggttcagaaggtgttcttgaacttcatcccattttttt

SEQ ID NO: 37 - DNA, 401 bp, synthetic construct
  source 1..401: mol_type = other DNA
gagggcctatttcccatgattccttcatatttgcatatacgatacaaggctgttagagagataattggaattaatttgactgtaaacacaaagatattagtacaaaatacgtgacgtagaaagtaataatttcttgggtagtttgcagttttaaaattatgttttaaaatggactatcatatgcttaccgtaacttgaaagtatttcgatttcttggctttatatatcttgtggaaaggacgaaacaccgccgggcatggtggcgcacgcctttaatcatttcttggtttctgtgatattctattggattgcatctactgaatagggacccaccttccaacatttcattcaacagttgcctccggttcagaaggtgttcttgaacttcatcccattttttt

SEQ ID NO: 38 - DNA, 56 bp, synthetic construct
  source 1..56: mol_type = other DNA
gagccacacttggacaggacgttgctaagaaccagcttcttattatttatctgcac

SEQ ID NO: 39 - DNA, 344 bp, synthetic construct
  source 1..344: mol_type = other DNA
gagggcctatttcccatgattccttcatatttgcatatacgatacaaggctgttagagagataattggaattaatttgactgtaaacacaaagatattagtacaaaatacgtgacgtagaaagtaataatttcttgggtagtttgcagttttaaaattatgttttaaaatggactatcatatgcttaccgtaacttgaaagtatttcgatttcttggctttatatatcttgtggaaaggacgaaacaccgccggtagtggtggcgcacgccggtaggatttgagccacacttggacaggacgttgctaagaaccagcttcttattatttatctgcacttttttt

SEQ ID NO: 40 - DNA, 3191 bp, synthetic construct
  source 1..3191: mol_type = other DNA
tgacgataaaggatcgtgaacctccaaaatcaggggatcgcagcggctacagcagccccggctccccaggcactcccggcagccgctcccgcaccccgtcccttccaaccccacccacccgggagcccaagaaggtggcagtggtccgtactccacccaagtcgccgtcttccgccaagagccgcctgcagacagcccccgtgcccatgccagacctgaagaatgtcaagtccaagatcggctccactgagaacctgaagcaccagccgggaggcgggaaggtgagagtggctggctgcgcgtggaggtgtggggggctgcgcctggaggggtagggctgtgcctggaagggtagggctgcgcctggaggtgcgcggttgagcgtggagtcgtgggactgtgcatggaggtgtggggctccccgcacctgagcacccccgcataacaccccagtcccctctggaccctcttcaaggaagttcagttctttattgggctctccactacactgtgagtgccctcctcaggcgagagaacgttctggctcttctcttgccccttcagcccctgttaatcggacagagatggcagggctgtgtctccacggccggaggctctcatagtcagggcacccacagcggttccccacctgccttctgggcagaatacactgccacccataggtcagcatctccactcgtgggccatctgcttaggttgggttcctctggattctggggagattgggggttctgttttgatcagctgattcttctgggagcaagtgggtgctcgcgagctctccagcttcctaaaggtggagaagcacagacttcgggggcctggcctggatccctttccccattcctgtccctgtgcccctcgtctgggtgcgttagggctgacatacaaagcaccacagtgaaagaacagcagtatgcctcctcactagccaggtgtgggcgggtgggtttcttccaaggcctctctgtggccgtgggtagccacctctgtcctgcaccgctgcagtcttccctctgtgtgtgctcctggtagctctgcgcatgctcatcttcttataagaacaccatggcagctgggcgtagtggctcacgcctataatcccagcactttgggaggctgaggcaggcagatcacgaggtcaggagttcgagaccaacctgaccaacagggtgaaacctcgtctctactaaaaatacaaaaatacctgggcgtggtggtggtgcgcgcctataatcccagctactcaggaggctgaggcaggagaatcgcttgaacccaggaggcagaggttgcagtgagccgagatagtgccactgcactccagtttgagcaacagagcgagactctgtctcaaaacaaaataaaacaaaccaaaaaaacccaccatggcttagggcccagcctgatgacctcatttttcacttagtcacctctctaaaggccctgtctccaaatagagtcacattctaaggtacgggggtgttggggaggggggttagggcttcaacatgtgaatttgcggggaccacaattcagcccaggaccccgctcccgccacccagcactggggagctggggaagggtgaagaggaggctgggggtgagaaggaccacagctcactctgaggctgcagatgtgctgggccttctgggcactgggcctcggggagctagggggctttctggaaccctgggcctgcgtgtcagcttgcctcccccacgcaggcgctctccacaccattgaagttcttatcactcaggcttgagaacagccgcagggagttctctgggaatgtgccggtgggtctagccaggtgtgagtggagatgccggggaacttcctattactcactcgtcagtgtggccgaacacatttttcacttgacctcaggctggtgaacgctcccctctggggttcaggcctcacgatgccatccttttgtgaagtgaggacctgcaatcccagcttcgtaaagcccgctggaaatcactcacacttctgggatgccttcagagcagccctctatcccttcagctcccctgggatgtgactcaacctcccgtcactccccagactgcctctgccaagtccgaaagtggaggcatccttgcgagcaagtaggcgggtccagggtggcgcatgtcactcatcgaaagtggaggcgtccttgcgagcaagcaggcgggtccagggtggcgtgtcactcatccttttttctggctaccaaaggtgcagataattaataagaagctggatcttagcaacgtccagtccaagtgtggctcaaaggataatatcaaacacgtcccgggaggcggcagtgtgagtaccttcacacgtcccatgcgccgtgctgtggcttgaattattaggaagtggtgtgagtgcgtacacttgcgagacactgcatagaataaatccttcttgggctctcaggatctggctgcgacctctgggtgaatgtagcccggctccccacattcccccacacggtccactgttcccagaagccccttcctcatattctaggagggggtgtcccagcatttctgggtcccccagcctgcgcaggctgtgtggacagaatagggcagatgacggaccctctctccggaccctgcctgggaagctgagaatacccatcaaagtctccttccactcatgcccagccctgtccccaggagccccatagcccattggaagttgggctgaaggtggtggcacctgagatgtctgggtcttgcacaatgacaatgggtccctgtttttcccagaggctcttttgttctgcagggattgaagacactccagtcccacagtccccagctcccctggggcagggttggcagaatttcgacaacacatttttccaccctgactaggatgtgctcctcatggcagctgggaaccactgtccaataagggcctgggcttacacagctgcttctcattgagttacacccttaataaaataatcccattttatcctttttgtctctctgtcttcctctctctctgcctttcctcttctctctcctcctctctcatctccaggtgcaaatagtctacaaaccagttgacctgagcaaggtgacctccaagtgtggctcattaggcaacatccatcataaaccagtcgagcatgcatctatcgagcatgcatcta

SEQ ID NO: 41 - DNA, 30 bp, synthetic construct; identical to SEQ ID NO: 15
  source 1..30: mol_type = other DNA

SEQ ID NO: 42 - DNA, 25 bp, synthetic construct
  source 1..25: mol_type = other DNA
caactggtttgtagactatttgcac